European Patent Application EP 4 506 358 A1, published February 12, 2025. Title: ICOS-L variants with enhanced binding to ICOS. Applicant: Korea University Research and Business Foundation. Application KR. The sequence listing filed with the application follows.

SEQUENCE LISTING (8 sequences)

SEQ ID NO: 1 - protein, 238 aa, synthetic construct [sequence omitted]

SEQ ID NO: 2 - protein, 238 aa, synthetic construct
  source 1..238: note = Y8_P51Q
DTQEKEVRAMVGSDVELSCACPEGSRFDLNDVYVYWQTSESKTVVTYHIPQNSSLEHVDSRYRNRALMSPAGMLRGDFSLRLFNVTPQDEQKFHCLVLSQSLGFQEVLSVEVTLHVAANFSVPVVSAPHSPSQDELTFTCTSINGYPRPNVYWINKTDNSLLDQALQNDTVFLNMRGLYDVVSVLRIARTPSVNIGCCIENVLLQQNLTVGSQTGNDIGERDKITENPVSTGEKNAAT

SEQ ID NO: 3 - protein, 238 aa, synthetic construct
  source 1..238: note = Y8_H57N
DTQEKEVRAMVGSDVELSCACPEGSRFDLNDVYVYWQTSESKTVVTYHIPPNSSLENVDSRYRNRALMSPAGMLRGDFSLRLFNVTPQDEQKFHCLVLSQSLGFQEVLSVEVTLHVAANFSVPVVSAPHSPSQDELTFTCTSINGYPRPNVYWINKTDNSLLDQALQNDTVFLNMRGLYDVVSVLRIARTPSVNIGCCIENVLLQQNLTVGSQTGNDIGERDKITENPVSTGEKNAAT

SEQ ID NO: 4 - protein, 238 aa, synthetic construct
  source 1..238: note = Y8
DTQEKEVRAMVGSDVELSCACPEGSRFDLNDVYVYWQTSESKTVVTYHIPPNSSLEHVDSRYRNRALMSPAGMLRGDFSLRLFNVTPQDEQKFHCLVLSQSLGFQEVLSVEVTLHVAANFSVPVVSAPHSPSQDELTFTCTSINGYPRPNVYWINKTDNSLLDQALQNDTVFLNMRGLYDVVSVLRIARTPSVNIGCCIENVLLQQNLTVGSQTGNDIGERDKITENPVSTGEKNAAT

SEQ ID NO: 5 - protein, 238 aa, synthetic construct
  source 1..238: note = Y13
DTQEKEVRAMVGSDVELSCACPEGSRFDLNDVYVYWQTSESKTVVTYHIPHNSNLENVDSRYRNRALMSPAGMLRGDFSLRLFNVTPQDEQKFHCLVLSQSLGFQEVLSVEVTLHVAANFSVPVVSAPHCPSQDELTFTCTSINGYPRPNVYWINKTDNSLLDQALQNDTVFLNMRGLYDVVSVLRIARTPSVNIGCCIENVLLQQNLTVGSQTGNDIGERDKITENPVSTGEKNAAT

SEQ ID NO: 6 - protein, 238 aa, synthetic construct
  source 1..238: note = Y20
DTQEKEVRAMVGSDVELSCACPEGSRFDLNDVYVYWQTSESKTVVTYHIPQSSSLENVDSRYRNRALMSPAGMLRGDFSLRLFNVTPQDEQKFHCLVLSQSLGFQEVLSVEVTLHVAANFSVPVVSAPHSPSQDELTFTCTSINGYPRPNVYWINKTDNSLLDQALQNDTVFLNMRGLYDVVSVLRIARTPSVNIGCCIENVLLQQNLTVGSQTGNDIGERDKITENPVSTGERNAAT

SEQ ID NO: 7 - protein, 238 aa, synthetic construct
  source 1..238: note = Y35
DTQDKEVRAMVGSDVELSCACPEGSRFDLNDVYVYWQTSESKTVVTYHIPPNSSLENVDSRYRNRALMSPAGMLRGDFSLRLFNVTPQDEQKFHCLVLSQSLGFQEVLSVEVTLHVAANFSVPVVSAPHSPSQDELTFTCTSINGYPRPNVYWINKTDNSLLDQALQNDTVFLNMRGLYDVVSVLRIARTPSVNIGCCIENVLLQQNLTVGSQTGNDIGERDKITENPVSTGEKNAAT

SEQ ID NO: 8 - protein, 238 aa, synthetic construct
  source 1..238: note = Y48
DTQEKEVRAMVGSDVELSCACPEGSRFDLNDVYVYWQTSESKTVVTYHIPPNSSLENVDSRYRNRALMSPAGMRRGDFSLRLFNVTPQDEQKFHCLVLSQSLGFQEVLSVEVTLHVAANFSVPVVSAPHSPSQDELTFTCTSINGYPRPNVYWINKTDNSLLDQALQNDTVFLNMRGLYDVVSVLRIARTPSVNIGCCIENVLLQQNLTVGSQTGNDIGERDKITENPVSTGEKNAAT